European Patent Application EP 4 501 910 A1, published February 5, 2025. Title: NITROGEN-CONTAINING HETEROCYCLIC COMPOUNDS AND THEIR USES. Applicant: BnH Research Co.,Ltd. The sequence listing filed with the application follows.

SEQUENCE LISTING (6 sequences)

SEQ ID NO: 1 - DNA, 20 bp, synthetic construct
  source 1..20: mol_type = other DNA; note = h-GluN2B-forward primer
cttccatttaccctgcctca

SEQ ID NO: 2 - DNA, 20 bp, synthetic construct
  source 1..20: mol_type = other DNA; note = h-GluN2B-reverse primer
cattgcctctagctcccttg

SEQ ID NO: 3 - DNA, 22 bp, synthetic construct
  source 1..22: mol_type = other DNA; note = h-BDNF-forward primer
catccgaggacaaggtggcttg

SEQ ID NO: 4 - DNA, 22 bp, synthetic construct
  source 1..22: mol_type = other DNA; note = h-BDNF-reverse primer
gccgaactttctggtcctcatc

SEQ ID NO: 5 - DNA, 18 bp, synthetic construct
  source 1..18: mol_type = other DNA; note = h-ActinB-forward primer
caccaactgggacgacat

SEQ ID NO: 6 - DNA, 18 bp, synthetic construct
  source 1..18: mol_type = other DNA; note = h-ActinB-reverse primer
acagcctggatagcaacg